European Patent Application EP 4 119 661 A1, published January 18, 2023. Title: PHYTASE VARIANTS WITH IMPROVED STABILITY AND IP4 ACTIVITY ( en ). Applicant: AB enzymes. The sequence listing filed with the application follows.

SEQUENCE LISTING (5 sequences)

SEQ ID NO: 1 - protein, 410 aa, Escherichia coli
QSEPELKLESVVIVSRHGVRAPTKFTQLMQDVTPDAWPTWPVKLGELTPRGGELIAYLGHYWRQRLVADGLLPKEGCPQSGQVAIIADVDERTRKTGEAFAAGLAPDCAITVHHQADTSSPDPLFNPLKTGVCQLDVANVRRAILERAGGSIADFTRHYQTAFRELERVLNFPQSNLCLKREKQDESCSLTQALPSELKVSADDVSLTGAWSLASMLTEIFLLQQAQGMPEPGWGRITDSHQWNTLLSLHNAVFDLLQRTPEVARSRATPLLDLIKTALTPHPPQKQAYGVTLPTSVLFIAGHDTNLANLGGALELNWTLPGQPDNYPPGGELVFERWRRLSDNSQWIQVSLVFQTLQQMRDKTPLSLNTPPGEVKLTLAGCEERNAQGMCSLAGFTQIVNEARIPACSL

SEQ ID NO: 2 - protein, 410 aa, Escherichia coli
QSEPELKLESVVIVSRHGVRAPTKFTQLMRDVTPDAWPTWPVKLGELTPRGGELIAYLGHYWRQRLVADGLLPKEGCPQPGQVAIIADVDERTLKTGEAFAAGLAPDCAITVHHQADLSSKDPLFHPLKTGVCQLDVANVRRAILERAGGSIADFTRHYQTAFRELERVLNFPQSPLCKNREAQDESCSLTQALPSELKVSADNVSLTGAVGLASTLTEIFLLEQAEGMPEPGWGRITDSHQWNTLLSLHNAYFDLLQRTPEVARSRATPLLDLIMAALTPHPPQKSAYGVTLPTSVLFIAGHDTNLANLGGALGLNWTLPGQPDNYPPGGELVFERWRRLSDNSQWIQVSMVFQTLQQMRDKTPLSLNTPPGEVKLTLPGCEERNAQGMCSLAGFTQIVNEARIPACSL

SEQ ID NO: 3 - protein, 410 aa, Escherichia coli
QSEPELKLESVVIVSRHGVRAPTKFTQLMRDVTPDAWPTWPVKLGELTPRGGELIAYLGHYWRQRLVADGLLPKEGCPQPGQVAIIADVDERTLKTGEAFAAGLAPDCAITVHHQADLSSPDPLFHPLKTGVCQLDVANVRRAILERAGGSIADFTRHYQTAFRELERVLNFPQSPLCKNREAQDESCSLTQALPSELKVSADNVSLTGAVGLASTLTEIFLLEQAEGMPEPGWGRITDSHQWNTLLSLHNAYFDLLQRTPEVARSRATPLLDLIMAALTPHPPQKSAYGVTLPTSVLFIAGHDTNLANLGGALGLNWTLPGQPDNYPPGGELVFERWRRLSDNSQWIQVSMVFQTLQQMRDKTPLSLNTPPGEVKLTLPGCEERNAQGMCSLAGFTQIVNEARIPACSL

SEQ ID NO: 4 - protein, 410 aa, Escherichia coli
QSEPELKLESVVIVSRHGVRAPTKFTQLMRDVTPDAWPTWPVKLGELTPRGGELISYLGHYWRQRLIADGLLPKEGCPQPGQVAIIADVDERTLKTGEAFAAGLAPNCAITVHHQADLSSKDPLFHPLKTGVCQLDVANVRRAILERAGGSIANFTRHYQTAFRELERVLNFPESPLCKNREKQDESCSLTQALPSELKVSSDNVSLTGAVGLASMLTEIFLLEQAEGMPEPGWGRITDSHQWNTLLSLHNAYFDLLQRTPEVARSRATPILDLIMAALTPHPPEKSAYGVTLPTSVLFIAAHDTNLANLGGALGLNWTLPGQPDNYPPGGELVFERWRRLSDDSQWIQVSMVFQTLQQMRDKTPLSLNTPPGEVKLTLPGCEERNAQGMCSLAAFTQIVNEARIPACSL

SEQ ID NO: 5 - protein, 410 aa, Escherichia coli
QSEPELKLESVVIVSRHGVRAPTKFTQLMRDVTPDAWPTWPVKLGELTPRGGELISYLGHYWRQRLIADGLLPKEGCPQPGQVAIIADVDERTLKTGEAFAAGLAPNCAITVHHQADLSSPDPLFHPLKTGVCQLDVANVRRAILERAGGSIANFTRHYQTAFRELERVLNFPESPLCKNREKQDESCSLTQALPSELKVSSDNVSLTGAVGLASTLTEIFLLEQAEGMPEPGWGRITDSHQWNTLLSLHNAYFDLLQRTPEVARSRATPILDLIMAALTPHPPEKSAYGVTLPTSVLFIAAHDTNLANLGGALGLNWTLPGQPDNYPPGGELVFERWRRLSDDSQWIQVSMVFQTLQQMRDKTPLSLNTPPGEVKLTLPGCEERNAQGMCSLAAFTQIVNEARIPACSL